European Patent Specification EP 3 478 325 B1, published July 17, 2024. Title: ELIMINATION OF PROLIFERATING CELLS FROM STEM CELL-DERIVED GRAFTS. Applicant: RESEARCH DEVELOPMENT FOUNDATION. The sequence listing filed with the application follows.

SEQUENCE LISTING (30 sequences)

SEQ ID NO: 1 - DNA, 21 bp, Artificial sequence
  Synthetic primer
gagcggtggttcgacaagtgg

SEQ ID NO: 2 - DNA, 19 bp, Artificial sequence
  Synthetic primer
cctcagcagggttggcatc

SEQ ID NO: 3 - DNA, 19 bp, Artificial sequence
  Synthetic primer
gatgccaaccctgctgagg

SEQ ID NO: 4 - DNA, 19 bp, Artificial sequence
  Synthetic primer
gtccagcctgtgctgggtg

SEQ ID NO: 5 - DNA, 19 bp, Artificial sequence
  Synthetic primer
cacccagcacaggctggac

SEQ ID NO: 6 - DNA, 21 bp, Artificial sequence
  Synthetic primer
cagggccacaaaagccagcac

SEQ ID NO: 7 - DNA, 21 bp, Artificial sequence
  Synthetic primer
gtgctggcttttgtggccctg

SEQ ID NO: 8 - DNA, 20 bp, Artificial sequence
  Synthetic primer
ccagagagctgtccccagtc

SEQ ID NO: 9 - DNA, 20 bp, Artificial sequence
  Synthetic primer
gtcccctgctggatgcagag

SEQ ID NO: 10 - DNA, 20 bp, Artificial sequence
  Synthetic primer
gtcccctgctggatgcagag

SEQ ID NO: 11 - DNA, 153 bp, Artificial sequence
  Synthetic oligonucleotide
atggcttcttaccctggacaccagcatgcttctgcctttgaccaggctgccagatccaggggccactccaacaggagaactgccctaagacccagaagacagcaggaagccactgaggtgaggcctgagcagaagatgccaaccctgctgagg

SEQ ID NO: 12 - DNA, 153 bp, Artificial sequence; identical to SEQ ID NO: 11
  Synthetic oligonucleotide

SEQ ID NO: 13 - DNA, 172 bp, Artificial sequence
  Synthetic oligonucleotide
gtgtacattgatggacctcatggcatgggcaagaccaccaccactcaactgctggtggcactgggctccagggatgacattgtgtatgtgcctgagccaatgacctactggagagtgctaggagcctctgagaccattgccaacatctacaccacccagcacaggctggacc

SEQ ID NO: 14 - DNA, 171 bp, Artificial sequence
  Synthetic oligonucleotide
gtgtacattgatggacctcatggcatgggcaagaccaccaccactcaactgctggtggcactgggctccagggatgacattgtgtatgtgcctgagccaatgacctactggagagtgctaggacctctgagaccattgccaacatctacaccacccagcacaggctggacc

SEQ ID NO: 15 - DNA, 233 bp, Artificial sequence
  Synthetic oligonucleotide
agggagaaatctctgctggagatgctgctgtggtgatgacctctgcccagatcacaatgggaatgccctatgctgtgactgatgctgttctggctcctcacattggaggagaggctggctcttctcatgcccctccacctgccctgaccctgatctttgacagacaccccattgcagccctgctgtgctacccagcagcaaggtacctcatgggctccatgaccccacaggct

SEQ ID NO: 16 - DNA, 233 bp, Artificial sequence; identical to SEQ ID NO: 15
  Synthetic oligonucleotide

SEQ ID NO: 17 - DNA, 232 bp, Artificial sequence
  Synthetic oligonucleotide
gtgctggcttttgtggccctgatccctccaaccctccctggcaccaacattgttctgggagcactgcctgaagacagacacattgacaggctggcaaagaggcagagacctggagagagactggacctggccatgctggctgcaatcagaagggtgtatggactgctggcaaacactgtgagatacctccagtgtggaggctcttggagagaggactggggacagctctctg

SEQ ID NO: 18 - DNA, 232 bp, Artificial sequence; identical to SEQ ID NO: 17
  Synthetic oligonucleotide

SEQ ID NO: 19 - DNA, 150 bp, Artificial sequence
  Synthetic oligonucleotide
atgctctgctgcaactaacctctggcatggtgcagacccatgtgaccacccctggcagcatccccaccatctgtgacctagccagaacctttgccagggagatgggaatctctggagccaatggagtcatggccaagttgaccagtgctg

SEQ ID NO: 20 - DNA, 150 bp, Artificial sequence; identical to SEQ ID NO: 19
  Synthetic oligonucleotide

SEQ ID NO: 21 - DNA, 111 bp, Artificial sequence
  Synthetic oligonucleotide
ggctggcacaggtagaaatctctgctggagatgctgctgtggtgatgacctctgcccagatcacaatgggaatgccctatgctgtgactgatgctgttctggctcctcaca

SEQ ID NO: 22 - DNA, 111 bp, Artificial sequence
  Synthetic oligonucleotide
ggctggcacagggagaaatctctgctggagatgctgctgtggtgatgacctctgcccagatcacaatgggaatgccctatgctgtgactgatgctgttctggctcctcaca

SEQ ID NO: 23 - DNA, 111 bp, Artificial sequence; identical to SEQ ID NO: 22
  Synthetic oligonucleotide

SEQ ID NO: 24 - DNA, 111 bp, Artificial sequence; identical to SEQ ID NO: 22
  Synthetic oligonucleotide

SEQ ID NO: 25 - DNA, 111 bp, Artificial sequence
  Synthetic oligonucleotide
ggctggcacagggagaaatctctgctggagatgctgctgtggtgatgacctctgcccagatcacaatgagaatgccctatgctgtgactgatgctgttctggctcctcaca

SEQ ID NO: 26 - DNA, 111 bp, Artificial sequence
  Synthetic oligonucleotide
ggctggcacagggagaaatctctgctggagatgctgctgtggtgatgacctctgcccagatcacaatgggaatgccctatgctgtgactgatgctgttctggttcctcaca

SEQ ID NO: 27 - protein, 13 aa, Artificial sequence
  Synthetic peptide
RVYIDGPHGMGKT

SEQ ID NO: 28 - protein, 13 aa, Artificial sequence
  Synthetic peptide
RVYIDGPHGMGKT

SEQ ID NO: 29 - DNA, 170 bp, Artificial sequence
  Synthetic oligonucleotide
gtcccctgctggatgcagagatgctctgctgcaactaacctctggcatggtgcagacccatgtgaccacccctggcagcatccccaccatctgtgacctagccagaacctttgccagggagatgggaatctctggagccaatggagtcatggccaagttgaccagtgctg

SEQ ID NO: 30 - DNA, 170 bp, Artificial sequence; identical to SEQ ID NO: 29
  Synthetic oligonucleotide